European Patent Application EP 4 321 518 A1, published February 14, 2024. Title: New polyphenol compound. Applicant: NABOCUL Cosmetics Co., Ltd. The sequence listing filed with the application follows.

SEQUENCE LISTING (2 sequences)

SEQ ID NO: 1 - DNA, 20 bp, Artificial Sequence
  Forward primer
tctgcgacaacggcaaggtg

SEQ ID NO: 2 - DNA, 20 bp, Artificial Sequence
  Reverse primer
gacgccggtggtttcttggt